European Patent Specification EP 3 722 308 B1, published February 21, 2024. Title: SULFATION OF WNT PATHWAY PROTEINS. Applicant: Enzo Biochem Inc. The sequence listing filed with the application follows.

SEQUENCE LISTING (27 sequences)

SEQ ID NO: 1 - protein, 12 aa, Homo sapiens
LGEYPEPPPELE

SEQ ID NO: 2 - protein, 8 aa, Homo sapiens
YVTDGPCR

SEQ ID NO: 3 - protein, 10 aa, Homo sapiens
ANQAELENAY

SEQ ID NO: 4 - protein, 16 aa, Homo sapiens
ELGEYPEPPPELENNK

SEQ ID NO: 5 - protein, 16 aa, Mus sp.
GLGEYPEPPPENNQTM

SEQ ID NO: 6 - protein, 16 aa, Rattus sp.
GLREYPEPPQELENNQ

SEQ ID NO: 7 - protein, 14 aa, Homo sapiens
ELGEYPEPPPELEN

SEQ ID NO: 8 - protein, 11 aa, Homo sapiens
KANQAELENAY

SEQ ID NO: 9 - protein, 13 aa, Homo sapiens
ELGEYPEPPPELE

SEQ ID NO: 10 - DNA, 20 bp, Artificial Sequence
  source 1..20: /mol_type="unassigned DNA" /note="Description of Artificial Sequence: Synthetic primer" /organism="Artificial Sequence"
caggggtggcaggcgttcaa

SEQ ID NO: 11 - DNA, 20 bp, Artificial Sequence
  source 1..20: /mol_type="unassigned DNA" /note="Description of Artificial Sequence: Synthetic primer" /organism="Artificial Sequence"
gtaggcgttctccagctcgg

SEQ ID NO: 12 - protein, 9 aa, Homo sapiens
IIYHMDEEE

SEQ ID NO: 13 - protein, 12 aa, Homo sapiens
DNYQPYPCAEDE

SEQ ID NO: 14 - protein, 9 aa, Mus sp.
DLDNYQPYP

SEQ ID NO: 15 - protein, 12 aa, Homo sapiens
GNNFDYWKYGEA

SEQ ID NO: 16 - protein, 11 aa, Homo sapiens
PDYWKYGEASS

SEQ ID NO: 17 - protein, 16 aa, Homo sapiens
ITSHDYLGQETLTEIQ

SEQ ID NO: 18 - protein, 15 aa, Mus sp.
IADHDYLGQETSTEV

SEQ ID NO: 19 - protein, 11 aa, Homo sapiens
AIAIDYDPLEG

SEQ ID NO: 20 - protein, 16 aa, Homo sapiens
PHSQYLSAEDSCPPSP

SEQ ID NO: 21 - protein, 16 aa, Mus sp.
TSDVNYDSEPVPPPTP

SEQ ID NO: 22 - protein, 188 aa, Homo sapiens
WQAFKNDATEIIPELGEYPEPPPELENNKTMNRAENGGRPPHHPFETKDVSEYSCRELHFTRYVTDGPCRSAKPVTELVCSGQCGPARLLPNAIGRGKWWRPSGPDFRCIPDRYRAQRVQLLCPGGEAPRARKVRLVASCKCKRLTRFHNQSELKDFGTEAARPQKGRKPRPRARSAKANQAELENAY

SEQ ID NO: 23 - protein, 9 aa, Mus sp.
IIYHMDEEE

SEQ ID NO: 24 - protein, 12 aa, Mus sp.
DNYQPYPCAEDE

SEQ ID NO: 25 - protein, 11 aa, Mus sp.
AIAIDYDPLEG

SEQ ID NO: 26 - protein, 16 aa, Mus sp.
PHSQYLSAEDSCPPSP

SEQ ID NO: 27 - protein, 4 aa, Unknown
  Description of Unknown: YWTD domain peptide
YWTD